European Patent Application EP 4 238 988 A1, published September 6, 2023. Title: ANTIBODIES AGAINST SARS-CoV-2 AND USES THEREOF. Applicant: CONSEJO SUPERIOR DE INVESTIGACIONES CIENTÍFICAS. The sequence listing filed with the application follows.

SEQUENCE LISTING (35 sequences)

SEQ ID NO: 1 - protein, 5 aa, Artificial Sequence
  VH-CDR1
DYNMH

SEQ ID NO: 2 - protein, 17 aa, Artificial Sequence
  VH-CDR2
YIYPYNGGTGYNQKFKS

SEQ ID NO: 3 - protein, 11 aa, Artificial Sequence
  VH-CDR3
AITTDYYAMDY

SEQ ID NO: 4 - protein, 15 aa, Artificial Sequence
  VL-CDR1
RASESVDNYGISFMN

SEQ ID NO: 5 - protein, 7 aa, Artificial Sequence
  VL-CDR2
AASNQGS

SEQ ID NO: 6 - protein, 9 aa, Artificial Sequence
  VL-CDR3
QQSKEVPWT

SEQ ID NO: 7 - protein, 30 aa, Artificial Sequence
  VH-FR1
EVQLQQSGPELVKPGASVKISCKASGYTFT

SEQ ID NO: 8 - protein, 14 aa, Artificial Sequence
  VH-FR2
WVKQSHGKSLEWIG

SEQ ID NO: 9 - protein, 32 aa, Artificial Sequence
  VH-FR3
KATLTVDNSSSTAYMELRSLTSEESAVYYCAR

SEQ ID NO: 10 - protein, 11 aa, Artificial Sequence
  VH-FR4
WGQGTSVTVSS

SEQ ID NO: 11 - protein, 23 aa, Artificial Sequence
  VL-FR1
DIVLTQSPASLAVSLGQRATISC

SEQ ID NO: 12 - protein, 15 aa, Artificial Sequence
  VL-FR2
WFQQKPGQAPKLLIY

SEQ ID NO: 13 - protein, 32 aa, Artificial Sequence
  VL-FR3
GVPARFSGSGSGTDFSLNIHPMEEDDTAMYFC

SEQ ID NO: 14 - protein, 10 aa, Artificial Sequence
  VL-FR4
FGGGTKVEIK

SEQ ID NO: 15 - protein, 575 aa, Artificial Sequence
  VH (sin  signal sequence)
EVQLQQSGPELVKPGASVKISCKASGYTFTDYNMHWVKQSHGKSLEWIGYIYPYNGGTGYNQKFKSKATLTVDNSSSTAYMELRSLTSEESAVYYCARAITTDYYAMDYWGQGTSVTVSSESQSFPNVFPLVSCESPLSDKNLVAMGCLARDFLPSTISFTWNYQNNTEVIQGIRTFPTLRTGGKYLATSQVLLSPKSILEGSDEYLVCKIHYGGKNRDLHVPIPAVAEMNPNVNVFVPPRDGFSGPAPRKSKLICEATNFTPKPITVSWLKDGKLVESGFTTDPVTIENKGSTPQTYKVISTLTISEIDWLNLNVYTCRVDHRGLTFLKNVSSTCAASPSTDILTFTIPPSFADIFLSKSANLTCLVSNLATYETLNISWASQSGEPLETKIKIMESHPNGTFSAKGVASVCVEDWNNRKEFVCTVTHRDLPSPQKKFISKPNEVHKHPPAVYLLPPAREQLNLRESATVTCLVKGFSPADISVQWLQRGQLLPQEKYVTSAPMPEPGAPGFYFTHSILTVTEEEWNSGETYTCVVGHEALPHLVTERTVDKSTGKPTLYNVSLIMSDTGGTCY

SEQ ID NO: 16 - protein, 218 aa, Artificial Sequence
  VL (sin  signal sequence)
DIVLTQSPASLAVSLGQRATISCRASESVDNYGISFMNWFQQKPGQAPKLLIYAASNQGSGVPARFSGSGSGTDFSLNIHPMEEDDTAMYFCQQSKEVPWTFGGGTKVEIKRADAAPTVSIFPPSSEQLTSGGASVVCFLNNFYPKDINVKWKIDGSERQNGVLNSWTDQDSKDSTYSMSSTLTLTKDEYERHNSYTCEATHKTSTSPIVKSFNRNEC

SEQ ID NO: 17 - protein, 223 aa, Artificial Sequence
  RBD1_CNB_WUHAN
RVQPTESIVRFPNITNLCPFGEVFNATRFASVYAWNRKRISNCVADYSVLYNSASFSTFKCYGVSPTKLNDLCFTNVYADSFVIRGDEVRQIAPGQTGKIADYNYKLPDDFTGCVIAWNSNNLDSKVGGNYNYLYRLFRKSNLKPFERDISTEIYQAGSTPCNGVEGFNCYFPLQSYGFQPTNGVGYQPYRVVVLSFELLHAPATVCGPKKSTNLVKNKCVNF

SEQ ID NO: 18 - protein, 223 aa, Artificial Sequence
  RBD1 (Lineage B.1.1.7 / Variant of Concern Alpha)
RVQPTESIVRFPNITNLCPFGEVFNATRFASVYAWNRKRISNCVADYSVLYNSASFSTFKCYGVSPTKLNDLCFTNVYADSFVIRGDEVRQIAPGQTGKIADYNYKLPDDFTGCVIAWNSNNLDSKVGGNYNYLYRLFRKSNLKPFERDISTEIYQAGSTPCNGVEGFNCYFPLQSYGFQPTYGVGYQPYRVVVLSFELLHAPATVCGPKKSTNLVKNKCVNF

SEQ ID NO: 19 - protein, 223 aa, Artificial Sequence
  RBD1 (lineages B.1.1.318/B.1.525/B.1.526)
RVQPTESIVRFPNITNLCPFGEVFNATRFASVYAWNRKRISNCVADYSVLYNSASFSTFKCYGVSPTKLNDLCFTNVYADSFVIRGDEVRQIAPGQTGKIADYNYKLPDDFTGCVIAWNSNNLDSKVGGNYNYLYRLFRKSNLKPFERDISTEIYQAGSTPCNGVKGFNCYFPLQSYGFQPTNGVGYQPYRVVVLSFELLHAPATVCGPKKSTNLVKNKCVNF

SEQ ID NO: 20 - protein, 223 aa, Artificial Sequence
  RBD1_CNB_SA (Beta, lineage B.1.351)
RVQPTESIVRFPNITNLCPFGEVFNATRFASVYAWNRKRISNCVADYSVLYNSASFSTFKCYGVSPTKLNDLCFTNVYADSFVIRGDEVRQIAPGQTGNIADYNYKLPDDFTGCVIAWNSNNLDSKVGGNYNYLYRLFRKSNLKPFERDISTEIYQAGSTPCNGVKGFNCYFPLQSYGFQPTYGVGYQPYRVVVLSFELLHAPATVCGPKKSTNLVKNKCVNF

SEQ ID NO: 21 - protein, 234 aa, Artificial Sequence
  RBD1_CNB_LA (Epsilon, California, lineage B.1.429)
ENLYFQGRVQPTESIVRFPNITNLCPFGEVFNATRFASVYAWNRKRISNCVADYSVLYNSASFSTFKCYGVSPTKLNDLCFTNVYADSFVIRGDEVRQIAPGQTGKIADYNYKLPDDFTGCVIAWNSNNLDSKVGGNYNYRYRLFRKSNLKPFERDISTEIYQAGSTPCNGVKGFNCLREKYFPLQSYGFQPTYGVGYQPYRVVVLSFELLHAPATVCGPKKSTNLVKNKCVNF

SEQ ID NO: 22 - protein, 223 aa, Artificial Sequence
  RBD1 (Kappa, India, B.1.617.1)
RVQPTESIVRFPNITNLCPFGEVFNATRFASVYAWNRKRISNCVADYSVLYNSASFSTFKCYGVSPTKLNDLCFTNVYADSFVIRGDEVRQIAPGQTGKIADYNYKLPDDFTGCVIAWNSNNLDSKVGGNYNYRYRLFRKSNLKPFERDISTEIYQAGSTPCNGVQGFNCYFPLQSYGFQPTNGVGYQPYRVVVLSFELLHAPATVCGPKKSTNLVKNKCVNF

SEQ ID NO: 23 - protein, 223 aa, Artificial Sequence; identical to SEQ ID NO: 22
  RBD1 (Delta, India, B.1.617.2)

SEQ ID NO: 24 - protein, 223 aa, Artificial Sequence
  RBD1 (B.1.620 )
RVQPTESIVRFPNITNLCPFGEVFNATRFASVYAWNRKRISNCVADYSVLYNSASFSTFKCYGVSPTKLNDLCFTNVYADSFVIRGDEVRQIAPGQTGKIADYNYKLPDDFTGCVIAWNSNNLDSKVGGNYNYLYRLFRKSNLKPFERDISTEIYQAGNTPCNGVKGFNCYFPLQSYGFQPTNGVGYQPYRVVVLSFELLHAPATVCGPKKSTNLVKNKCVNF

SEQ ID NO: 25 - protein, 223 aa, Artificial Sequence
  RBD1_CNB_BR (Lineage P.1, Brazil)
RVQPTESIVRFPNITNLCPFGEVFNATRFASVYAWNRKRISNCVADYSVLYNSASFSTFKCYGVSPTKLNDLCFTNVYADSFVIRGDEVRQIAPGQTGTIADYNYKLPDDFTGCVIAWNSNNLDSKVGGNYNYLYRLFRKSNLKPFERDISTEIYQAGSTPCNGVKGFNCYFPLQSYGFQPTYGVGYQPYRVVVLSFELLHAPATVCGPKKSTNLVKNKCVNF

SEQ ID NO: 26 - protein, 223 aa, Artificial Sequence
  P.3 (Theta)
RVQPTESIVRFPNITNLCPFGEVFNATRFASVYAWNRKRISNCVADYSVLYNSASFSTFKCYGVSPTKLNDLCFTNVYADSFVIRGDEVRQIAPGQTGKIADYNYKLPDDFTGCVIAWNSNNLDSKVGGNYNYLYRLFRKSNLKPFERDISTEIYQAGSTPCNGVKGFNCYFPLQSYGFQPTYGVGYQPYRVVVLSFELLHAPATVCGPKKSTNLVKNKCVNF

SEQ ID NO: 27 - protein, 223 aa, Artificial Sequence
  RBD1 (Omicron, B.1.1.529)
RVQPTESIVRFPNITNLCPFDEVFNATRFASVYAWNRKRISNCVADYSVLYNLAPFFTFKCYGVSPTKLNDLCFTNVYADSFVIRGDEVRQIAPGQTGNIADYNYKLPDDFTGCVIAWNSNKLDSKVSGNYNYLYRLFRKSNLKPFERDISTEIYQAGNKPCNGVAGFNCYFPLRSYSFRPTYGVGHQPYRVVVLSFELLHAPATVCGPKKSTNLVKNKCVNF

SEQ ID NO: 28 - protein, 223 aa, Artificial Sequence
  RBD1 (C.37, Lambda, Perú)
RVQPTESIVRFPNITNLCPFGEVFNATRFASVYAWNRKRISNCVADYSVLYNSASFSTFKCYGVSPTKLNDLCFTNVYADSFVIRGDEVRQIAPGQTGKIADYNYKLPDDFTGCVIAWNSNNLDSKVGGNYNYQYRLFRKSNLKPFERDISTEIYQAGSTPCNGVEGFNCYSPLQSYGFQPTNGVGYQPYRVVVLSFELLHAPATVCGPKKSTNLVKNKCVNF

SEQ ID NO: 29 - protein, 223 aa, Artificial Sequence
  RBD1 (B.1.621, Mu, Colombia)
RVQPTESIVRFPNITNLCPFGEVFNATKFASVYAWNRKRISNCVADYSVLYNSASFSTFKCYGVSPTKLNDLCFTNVYADSFVIRGDEVRQIAPGQTGKIADYNYKLPDDFTGCVIAWNSNNLDSKVGGNYNYLYRLFRKSNLKPFERDISTEIYQAGSTPCNGVKGFNCYFPLQSYGFQPTYGVGYQPYRVVVLSFELLHAPATVCGPKKSTNLVKNKCVNF

SEQ ID NO: 30 - protein, 20 aa, Artificial Sequence
  signal peptide
MVSAIVLYVLLAAAAHSAFA

SEQ ID NO: 31 - protein, 9 aa, Artificial Sequence
  histidine tail
HHHHHHHHH

SEQ ID NO: 32 - DNA, 1785 bp, Artificial Sequence
  DNA encoding Heavy chain with signal sequence
atgggatggagctggatctttctcttcctcctgtcaggaactgcaggcgtccactctgaggtccagcttcagcagtcaggacctgagctggtgaaacctggggcctcagtgaagatatcctgcaaggcttctggatacacattcactgactacaacatgcactgggtgaagcagagccatggaaagagccttgagtggattggatatatttatccttacaatggtggtactggctacaaccagaagttcaagagcaaggccacattgactgtagacaattcctccagcacagcctacatggagctccgcagcctgacatctgaggagtctgcagtctattactgtgcaagagcgattacgacggattactatgctatggactactggggtcaaggaacctcagtcaccgtctcctcagagagtcagtccttcccaaatgtcttccccctcgtctcctgcgagagccccctgtctgataagaatctggtggccatgggctgcctggcccgggacttcctgcccagcaccatttccttcacctggaactaccagaacaacactgaagtcatccagggtatcagaaccttcccaacactgaggacagggggcaagtacctagccacctcgcaggtgttgctgtctcccaagagcatccttgaaggttcagatgaatacctggtatgcaaaatccactacggaggcaaaaacagagatctgcatgtgcccattccagctgtcgcagagatgaaccccaatgtaaatgtgttcgtcccaccacgggatggcttctctggccctgcaccacgcaagtctaaactcatctgcgaggccacgaacttcactccaaaaccgatcacagtatcctggctaaaggatgggaagctcgtggaatctggcttcaccacagatccggtgaccatcgagaacaaaggatccacaccccaaacctacaaggtcataagcacacttaccatctctgaaatcgactggctgaacctgaatgtgtacacctgccgtgtggatcacaggggtctcaccttcttgaagaacgtgtcctccacatgtgctgccagtccctccacagacatcctaaccttcaccatccccccctcctttgccgacatcttcctcagcaagtccgctaacctgacctgtctggtctcaaacctggcaacctatgaaaccctgaatatctcctgggcttctcaaagtggtgaaccactggaaaccaaaattaaaatcatggaaagccatcccaatggcaccttcagtgctaagggtgtggctagtgtttgtgtggaagactggaataacaggaaggaatttgtgtgtactgtgactcacagggatctgccttcaccacagaagaaattcatctcaaaacccaatgaggtgcacaaacatccacctgctgtgtacctgctgccaccagctcgtgagcaactgaacctgagggagtcagccacagtcacctgcctggtgaagggcttctctcctgcagacatcagtgtgcagtggcttcagagagggcaactcttgccccaagagaagtatgtgaccagtgccccgatgccagagcctggggccccaggcttctactttacccacagcatcctgactgtgacagaggaggaatggaactccggagagacctatacctgtgttgtaggccacgaggccctgccacacctggtgaccgagaggaccgtggacaagtccactggtaaacccacactgtacaatgtctccctgatcatgtctgacacaggcggcacctgctattga

SEQ ID NO: 33 - DNA, 717 bp, Artificial Sequence
  DNA encoding light chain with signal sequence
atggagaaagacacactcctgctatgggtcctgcttctctgggttccaggttccacaggtgacattgtgctgacccaatctccagcttctttggctgtgtctctagggcagagggccaccatctcctgcagagccagcgaaagtgttgataattatggcattagttttatgaactggttccaacagaaaccaggacaggcacccaaactcctcatctatgctgcatccaaccaaggatccggggtccctgccaggtttagtggcagtgggtctgggacagacttcagtctcaacatccatcctatggaggaggatgatactgcaatgtatttctgtcagcaaagtaaggaggttccgtggacgttcggtggaggcaccaaggtggaaatcaaacgggctgatgctgcaccaactgtatccatcttcccaccatccagtgagcagttaacatctggaggtgcctcagtcgtgtgcttcttgaacaacttctaccccaaagacatcaatgtcaagtggaagattgatggcagtgaacgacaaaatggcgtcctgaacagttggactgatcaggacagcaaagacagcacctacagcatgagcagcaccctcacgttgaccaaggacgagtatgaacgacataacagctatacctgtgaggccactcacaagacatcaacttcacccattgtcaagagcttcaacaggaatgagtgttag

SEQ ID NO: 34 - protein, 594 aa, Artificial Sequence
  VH (with signal sequence)
MGWSWIFLFLLSGTAGVHSEVQLQQSGPELVKPGASVKISCKASGYTFTDYNMHWVKQSHGKSLEWIGYIYPYNGGTGYNQKFKSKATLTVDNSSSTAYMELRSLTSEESAVYYCARAITTDYYAMDYWGQGTSVTVSSESQSFPNVFPLVSCESPLSDKNLVAMGCLARDFLPSTISFTWNYQNNTEVIQGIRTFPTLRTGGKYLATSQVLLSPKSILEGSDEYLVCKIHYGGKNRDLHVPIPAVAEMNPNVNVFVPPRDGFSGPAPRKSKLICEATNFTPKPITVSWLKDGKLVESGFTTDPVTIENKGSTPQTYKVISTLTISEIDWLNLNVYTCRVDHRGLTFLKNVSSTCAASPSTDILTFTIPPSFADIFLSKSANLTCLVSNLATYETLNISWASQSGEPLETKIKIMESHPNGTFSAKGVASVCVEDWNNRKEFVCTVTHRDLPSPQKKFISKPNEVHKHPPAVYLLPPAREQLNLRESATVTCLVKGFSPADISVQWLQRGQLLPQEKYVTSAPMPEPGAPGFYFTHSILTVTEEEWNSGETYTCVVGHEALPHLVTERTVDKSTGKPTLYNVSLIMSDTGGTCY

SEQ ID NO: 35 - protein, 238 aa, Artificial Sequence
  VL (with signal sequence)
MEKDTLLLWVLLLWVPGSTGDIVLTQSPASLAVSLGQRATISCRASESVDNYGISFMNWFQQKPGQAPKLLIYAASNQGSGVPARFSGSGSGTDFSLNIHPMEEDDTAMYFCQQSKEVPWTFGGGTKVEIKRADAAPTVSIFPPSSEQLTSGGASVVCFLNNFYPKDINVKWKIDGSERQNGVLNSWTDQDSKDSTYSMSSTLTLTKDEYERHNSYTCEATHKTSTSPIVKSFNRNEC